European Patent Specification EP 3 713 600 B1, published May 6, 2026. Title: SYNTHETIC HEMAGGLUTININ AS UNIVERSAL VACCINE AGAINST INFECTION BY TYPE B INFLUENZA VIRUSES (IBV). Applicant: Her Majesty the Queen in Right of Canada as Represented by the Minister of Health Li, Xugang Van Domselaar, Gary Zetner, Adrian. The sequence listing filed with the application follows.

SEQUENCE LISTING (5 sequences)

SEQ ID NO: 1 - protein, 223 aa, Influenza B virus
GFFGAIAGFLEGGWEGMIAGWHGYTSHGAHGVAVAADLKSTQEAINKITKNLNSLSELEVKNLQRLSGAMDELHNEILELDEKVDDLRADTISSQIELAVLLSNEGIINSEDEHLLALERKLKKMLGPSAVEIGNGCFETKHKCNQTCLDRIAAGTFNAGEFSLPTFDSLNITAASLNDDGLDNHTILLYYSTAASSLAVTLMLAIFIVYMVSRDNVSCSICL

SEQ ID NO: 2 - protein, 222 aa, Influenza B virus
  VARIANT (132)..(132): D or E
  VARIANT (158)..(158): N or D
  misc_feature (203)..(203): Xaa can be any naturally occurring amino acid
  VARIANT (204)..(204): I or L
  misc_feature (207)..(207): Xaa can be any naturally occurring amino acid
  VARIANT (208)..(208): I or V
  misc_feature (211)..(211): Xaa can be any naturally occurring amino acid
  VARIANT (212)..(212): V or I
GFFGAIAGFLEGGWEGMIAGWHGYTSHGAHGVAVAADLKSTQEAINKITKNLNSLSELEVKNLQRLSGAMDELHNEILELDEKVDDLRADTISSQIELAVLLSNEGIINSEDEHLLALERKLKKMLGPSAVXIGNGCFETKHKCNQTCLDRIAAGTFXAGEFSLPTFDSLNITASLNDDGLDNHTILLYYSTAASSLAVTLMXAIFXVYMXSRDNVSCSICL

SEQ ID NO: 3 - DNA, 669 bp, Influenza B virus
gggtttttcggcgccatcgccggcttcctggagggcggctgggagggcatgatcgccggctggcacggctacaccagccacggcgcccacggcgtggccgtggccgccgacctgaagagcacccaggaggccattaacaagatcacaaagaacctgaacagcctgtccgagctggaggtgaagaacctgcagaggctgagtggcgccatggatgagctgcacaacgagatcctggagctggacgagaaggtggatgacctgagggctgacaccatcagctctcagattgagctggccgtgctgctgtctaacgagggcatcatcaacagcgaggacgagcacctgctggccctggagagaaagctgaagaagatgctgggaccctccgccgtggagatcggaaacggctgctttgagaccaagcacaagtgcaaccagacctgtctggacagaatcgccgccggcaccttcaatgccggagagttcagcctgcccaccttcgacagcctgaacatcaccgccgctagcctgaacgacgacggactggacaaccacaccatcctgctgtactacagcacagccgccagctccctggccgtcaccctgatgctggccatcttcatcgtgtacatggtgagcagagataacgtgtcttgttccatctgcctg

SEQ ID NO: 4 - protein, 23 aa, artificial sequence
  Signal sequence peptide
MLLAVLYCLLWSFQTSAGHFPRA

SEQ ID NO: 5 - protein, 27 aa, artificial sequence
  trimerization motif peptide
YIPEAPRDGQAYVRKDGEWVLLSTFLG